European Patent Specification EP 3 901 283 B1, published August 6, 2025. Title: THERAPEUTIC TREATMENT OF BREAST CANCER BASED ON C-MAF STATUS. Applicant: InBioMotion S.L. COLEMAN, ROBERT E. GREGORY, WALTER GOMIS, ROGER TERCERO, JUAN CARLOS. The sequence listing filed with the application follows.

SEQUENCE LISTING (24 sequences)

SEQ ID NO: 1 - DNA, 6878 bp, Homo sapiens
agaggctttaaaatcttttttcatcttctagctgtagctcgggctgcttgtcggcttggcctccccctcccccctttgctctctgcctcgtctttccccaggacttcgctattttgcttttttaaaaaaaggcaagaaagaactaaactcccccctccctctcctccagtcgggctgcacctctgccttgcactttgcacagaggtagagagcgcgcgagggagagagaggaaagaaaaaaaataataaagagagccaagcagaagaggaggcgagaagcatgaagtgttaactcccccgtgccaaggcccgcgccgcccggacagacgcccgccgcgcctccagccccgagcggacgccgcgcgcgccctgcctgcagcccgggccggcgaggcgagcccttccttatgcaaagcgcgcagcggagcggcgagcgggggacgccgcgcaccgggccgggctcctccagcttcgccgccgcagccaccaccgccgccaccgcagctcgcggaggatcttcccgagcctgaagccgccggctcggcgcgcaaggaggcgagcgagcaaggaggggccggggcgagcgagggagcacattggcgtgagcaggggggagggagggcgggcgcggggggcgcgggcagggcgggggggtgtgtgtgtgagcgcgctcggaggtttcgggccagccaccgccgcgcaagctagaagcgccccagcccggcaagctggctcacccgctggccacccagcacagcccgctggcccctctcctgcagcccatctggcggagcggcggcggcggcggcggcggcggcaggagaatggcatcagaactggcaatgagcaactccgacctgcccaccagtcccctggccatggaatatgttaatgacttcgatctgatgaagtttgaagtgaaaaaggaaccggtggagaccgaccgcatcatcagccagtgcggccgtctcatcgccgggggctcgctgtcctccacccccatgagcacgccgtgcagctcggtgcccccttcccccagcttctcggcgcccagcccgggctcgggcagcgagcagaaggcgcacctggaagactactactggatgaccggctacccgcagcagctgaaccccgaggcgctgggcttcagccccgaggacgcggtcgaggcgctcatcagcaacagccaccagctccagggcggcttcgatggctacgcgcgcggggcgcagcagctggccgcggcggccggggccggtgccggcgcctccttgggcggcagcggcgaggagatgggccccgccgccgccgtggtgtccgccgtgatcgccgcggccgccgcgcagagcggcgcgggcccgcactaccaccaccaccaccaccacgccgccggccaccaccaccacccgacggccggcgcgcccggcgccgcgggcagcgcggccgcctcggccggtggcgctgggggcgcgggcggcggtggcccggccagcgctgggggcggcggcggcggcggcggcggcggaggcggcgggggcgcggcgggggcggggggcgccctgcacccgcaccacgccgccggcggcctgcacttcgacgaccgcttctccgacgagcagctggtgaccatgtctgtgcgcgagctgaaccggcagctgcgcggggtcagcaaggaggaggtgatccggctgaagcagaagaggcggaccctgaaaaaccgcggctatgcccagtcctgccgcttcaagagggtgcagcagagacacgtcctggagtcggagaagaaccagctgctgcagcaagtcgaccacctcaagcaggagatctccaggctggtgcgcgagagggacgcgtacaaggagaaatacgagaagttggtgagcagcggcttccgagaaaacggctcgagcagcgacaacccgtcctctcccgagtttttcatgtgagtctgacacgcgattccagctagccaccctgataagtgctccgcgggggtccggctcgggtgtgggcttgctagttctagagccatgctcgccaccacctcaccacccccacccccaccgagtttggcccccttggccccctacacacacacaaacccgcacgcacacaccacacacacacacacacacacacacacaccccacaccctgctcgagtttgtggtggtggtggctgttttaaactggggagggaatgggtgtctggctcatggattgccaatctgaaattctccataacttgctagcttgttttttttttttttttacacccccccgccccacccccggacttgcacaatgttcaatgatctcagcagagttcttcatgtgaaacgttgatcacctttgaagcctgcatcattcacatattttttcttcttcttccccttcagttcatgaactggtgttcattttctgtgtgtgtgtgtgttttattttgtttggatttttttttttaattttacttttagagcttgctgtgttgcccaccttttttccaacctccaccctcactccttctcaacccatctcttccgagatgaaagaaaaaaaaaagcaaagtttttttttcttctcctgagttcttcatgtgagattgagcttgcaaaggaaaaaaaaatgtgaaatgttatagacttgcagcgtgccgagttccatcgggttttttttttagcattgttatgctaaaatagagaaaaaaatcctcatgaaccttccacaatcaagcctgcatcaaccttctgggtgtgacttgtgagttttggccttgtgatgccaaatctgagagtttagtctgccattaaaaaaactcattctcatctcatgcattattatgcttgctactttgtcttagcaacaatgaactataactgtttcaaagactttatggaaaagagacattatattaataaaaaaaaaaagcctgcatgctggacatgtatggtataattattttttcctttttttttccttttggcttggaaatggacgttcgaagacttatagcatggcattcatacttttgttttattgcctcatgacttttttgagtttagaacaaaacagtgcaaccgtagagccttcttcccatgaaattttgcatctgctccaaaactgctttgagttactcagaacttcaacctcccaatgcactgaaggcattccttgtcaaagataccagaatgggttacacatttaacctggcaaacattgaagaactcttaatgttttctttttaataagaatgacgccccactttggggactaaaattgtgctattgccgagaagcagtctaaaatttattttttaaaaagagaaactgccccattatttttggtttgttttatttttattttatattttttggcttttggtcattgtcaaatgtggaatgctctgggtttctagtatataatttaattctagtttttataatctgttagcccagttaaaatgtatgctacagataaaggaatgttatagataaatttgaaagagttaggtctgtttagctgtagattttttaaacgattgatgcactaaattgtttactattgtgatgttaaggggggtagagtttgcaaggggactgtttaaaaaaagtagcttatacagcatgtgcttgcaacttaaatataagttgggtatgtgtagtctttgctataccactgactgtattgaaaaccaaagtattaagaggggaaacgcccctgtttatatctgtaggggtattttacattcaaaaatgtatgtttttttttcttttcaaaattaaagtatttgggactgaattgcactaagatataacctgcaagcatataatacaaaaaaaaattgcaaaactgtttagaacgctaataaaatttatgcagttataaaaatggcattactgcacagttttaagatgatgcagatttttttacagttgtattgtggtgcagaactggattttctgtaacttaaaaaaaaatccacagttttaaaggcaataatcagtaaatgttattttcagggactgacatcctgtctttaaaaagaaatgaaaagtaaatcttaccacaataaatataaaaaaatcttgtcagttacttttcttttacatattttgctgtgcaaaattgttttatatcttgagttactaactaaccacgcgtgttgttcctatgtgcttttctttcattttcaattctggttatatcaagaaaagaataatctacaataataaacggcatttttttttgattctgtactcagtttcttagtgtacagtttaactgggcccaacaacctcgttaaaagtgtaaaatgcatccttttctccagtggaaggattcctggaggaatagggagacagtaattcagggtgaaattataggctgttttttgaagtgaggaggctggccccatatactgattagcaatatttaatatagatgtaaattatgacctcatttttttctccccaaagttttcagttttcaaatgagttgagccataattgcccttggtaggaaaaacaaaacaaaacagtggaactaggcttcctgagcatggccctacacttctgatcaggagcaaagccatccatagacagaggagccggacaaatatggcgcatcagaggtggcttgcgcacatatgcattgaacggtaaagagaaacagcgcttgccttttcactaaagttgactatttttccttcttctcttacacaccgagattttcttgttagcaaggcctgacaagatttaacataaacatgacaaatcatagttgtttgttttgttttgcttttctctttaacactgaagatcatttgtcttaaataggaaaaagaaaatccactccttacttccatatttccaagtacatatctggtttaaactatgttatcaaatcatatttcaccgtgaatattcagtggagaacttctctacctggatgagctagtaatgatttcagatcatgctatccccagaaataaaagcaaaaaataatacctgtgtggaatataggctgtgctttgatttactggtatttaccccaaaataggctgtgtatgggggctgacttaaagatcccttggaaagactcaaaactaccttcactagtaggactcctaagcgctgacctatttttaaatgacacaaattcatgaaactaatgttacaaattcatgcagtttgcactcttagtcatcttcccctagcacaccaatagaatgttagacaaagccagcactgttttgaaaatacagccaaacacgatgacttttgttttgttttctgccgttcttaaaagaaaaaaagataatattgcaactctgactgaaagacttatttttaagaaaacaggttgtgtttggtgctgctaagttctggccagtttatcatctggccttcctgcctattttttacaaaacacgaagacagtgtgtaacctcgacattttgaccttcctttatgtgctagtttagacaggctcctgaatccacacttaattttgcttaacaaaagtcttaatagtaaacctcccctcatgagcttgaagtcaagtgttcttgacttcagatatttctttcctttttttttttttttcctcatcacaactaagagatacacaaactctgaagaagcagaaatggagagaatgcttttaacaaaaaagcatctgatgaaagattttaggcaaacattctcaaaataagagtgatattctggatgtagttattgcagttatctcatgacaaatgaggcctggattggaaggaaaatatagttgtgtagaattaagcattttgataggaatctacaaggtagttgaatataataagcaggtttgggcccccaaactttagaaaatcaaatgcaaaggtgctggcaaaaatgaggtttgagtggctggctgtaagagaaggttaactcctagtaaaaggcatttttagaaataacaattactgaaaactttgaagtatagtgggagtagcaaacaaatacatgttttttttttcttacaaagaactcctaaatcctgagtaagtgccattcattacaataagtctctaaatttaaaaaaaaaaaaatcatatgaggaaatctagctttcccctttacgctgcgtttgatctttgtctaaatagtgttaaaattcctttcattccaattacagaactgagcccactcgcaagttggagccatcagtgggatacgccacattttggaagccccagcatcgtgtacttaccagtgtgttcacaaaatgaaatttgtgtgagagctgtacattaaaaaaaatcatcattattattattatttgcagtcatggagaaccacctacccctgacttctgtttagtctcctttttaaataaaaattactgtgttagagaagaaggctattaaatgtagtagttaactatgcctcttgtctgggggtttcatagagaccggtaggaaagcgcactcctgcttttcgatttatggtgtgtgcaagtaaacaggtgcattgctttcaacctgccatactagttttaaaaattcactgaaattacaaagatacatatatatgcatatatataatggaaagtttcccggaatgcaacaattagcattttaaaatcatatataggcatgcacattctaaatagtactttttcatgcttcattgtttctctggcagataattttactaagaagaaaaatagatattcgactccccttccctaaacaaatccacgggcagaggctccagcggagccgagccccctggttttctcgtaggccctagacggtgttgcatttatcagtgatgtcaaacgtgctcatttgtcagacatagctgtaaatgaaaacaatgtgtggcaaaatacaaagtt

SEQ ID NO: 2 - DNA, 2656 bp, Homo sapiens
gaggctttaaaatcttttttcatcttctagctgtagctcgggctgcttgtcggcttggcctccccctcccccctttgctctctgcctcgtctttccccaggacttcgctattttgcttttttaaaaaaaggcaagaaagaactaaactcccccctccctctcctccagtcgggctgcacctctgccttgcactttgcacagaggtagagagcgcgcgagggagagagaggaaagaaaaaaaataataaagagagccaagcagaagaggaggcgagaagcatgaagtgttaactcccccgtgccaaggcccgcgccgcccggacagacgcccgccgcgcctccagccccgagcggacgccgcgcgcgccctgcctgcagcccgggccggcgaggcgagcccttccttatgcaaagcgcgcagcggagcggcgagcgggggacgccgcgcaccgggccgggctcctccagcttcgccgccgcagccaccaccgccgccaccgcagctcgcggaggatcttcccgagcctgaagccgccggctcggcgcgcaaggaggcgagcgagcaaggaggggccggggcgagcgagggagcacattggcgtgagcaggggggagggagggcgggcgcggggggcgcgggcagggcgggggggtgtgtgtgtgagcgcgctcggaggtttcgggccagccaccgccgcgcaagctagaagcgccccagcccggcaagctggctcacccgctggccacccagcacagcccgctggcccctctcctgcagcccatctggcggagcggcggcggcggcggcggcggcggcaggagaatggcatcagaactggcaatgagcaactccgacctgcccaccagtcccctggccatggaatatgttaatgacttcgatctgatgaagtttgaagtgaaaaaggaaccggtggagaccgaccgcatcatcagccagtgcggccgtctcatcgccgggggctcgctgtcctccacccccatgagcacgccgtgcagctcggtgcccccttcccccagcttctcggcgcccagcccgggctcgggcagcgagcagaaggcgcacctggaagactactactggatgaccggctacccgcagcagctgaaccccgaggcgctgggcttcagccccgaggacgcggtcgaggcgctcatcagcaacagccaccagctccagggcggcttcgatggctacgcgcgcggggcgcagcagctggccgcggcggccggggccggtgccggcgcctccttgggcggcagcggcgaggagatgggccccgccgccgccgtggtgtccgccgtgatcgccgcggccgccgcgcagagcggcgcgggcccgcactaccaccaccaccaccaccacgccgccggccaccaccaccacccgacggccggcgcgcccggcgccgcgggcagcgcggccgcctcggccggtggcgctgggggcgcgggcggcggtggcccggccagcgctgggggcggcggcggcggcggcggcggcggaggcggcgggggcgcggcgggggcggggggcgccctgcacccgcaccacgccgccggcggcctgcacttcgacgaccgcttctccgacgagcagctggtgaccatgtctgtgcgcgagctgaaccggcagctgcgcggggtcagcaaggaggaggtgatccggctgaagcagaagaggcggaccctgaaaaaccgcggctatgcccagtcctgccgcttcaagagggtgcagcagagacacgtcctggagtcggagaagaaccagctgctgcagcaagtcgaccacctcaagcaggagatctccaggctggtgcgcgagagggacgcgtacaaggagaaatacgagaagttggtgagcagcggcttccgagaaaacggctcgagcagcgacaacccgtcctctcccgagtttttcataactgagcccactcgcaagttggagccatcagtgggatacgccacattttggaagccccagcatcgtgtacttaccagtgtgttcacaaaatgaaatttgtgtgagagctgtacattaaaaaaaatcatcattattattattatttgcagtcatggagaaccacctacccctgacttctgtttagtctcctttttaaataaaaattactgtgttagagaagaaggctattaaatgtagtagttaactatgcctcttgtctgggggtttcatagagaccggtaggaaagcgcactcctgcttttcgatttatggtgtgtgcaagtaaacaggtgcattgctttcaacctgccatactagttttaaaaattcactgaaattacaaagatacatatatatgcatatatataatggaaagtttcccggaatgcaacaattagcattttaaaatcatatataggcatgcacattctaaatagtactttttcatgcttcattgtttctctggcagataattttactaagaagaaaaatagatattcgactccccttccctaaacaaatccacgggcagaggctccagcggagccgagccccctggttttctcgtaggccctagacggtgttgcatttatcagtgatgtcaaacgtgctcatttgtcagacatagctgtaaatgaaaacaatgtgtggcaaaatacaaagttaaaaaaaaaa

SEQ ID NO: 3 - DNA, 6887 bp, Homo sapiens
gaggctttaaaatcttttttcatcttctagctgtagctcgggctgcttgtcggcttggcctccccctcccccctttgctctctgcctcgtctttccccaggacttcgctattttgcttttttaaaaaaaggcaagaaagaactaaactcccccctccctctcctccagtcgggctgcacctctgccttgcactttgcacagaggtagagagcgcgcgagggagagagaggaaagaaaaaaaataataaagagagccaagcagaagaggaggcgagaagcatgaagtgttaactcccccgtgccaaggcccgcgccgcccggacagacgcccgccgcgcctccagccccgagcggacgccgcgcgcgccctgcctgcagcccgggccggcgaggcgagcccttccttatgcaaagcgcgcagcggagcggcgagcgggggacgccgcgcaccgggccgggctcctccagcttcgccgccgcagccaccaccgccgccaccgcagctcgcggaggatcttcccgagcctgaagccgccggctcggcgcgcaaggaggcgagcgagcaaggaggggccggggcgagcgagggagcacattggcgtgagcaggggggagggagggcgggcgcggggggcgcgggcagggcgggggggtgtgtgtgtgagcgcgctcggaggtttcgggccagccaccgccgcgcaagctagaagcgccccagcccggcaagctggctcacccgctggccacccagcacagcccgctggcccctctcctgcagcccatctggcggagcggcggcggcggcggcggcggcggcaggagaatggcatcagaactggcaatgagcaactccgacctgcccaccagtcccctggccatggaatatgttaatgacttcgatctgatgaagtttgaagtgaaaaaggaaccggtggagaccgaccgcatcatcagccagtgcggccgtctcatcgccgggggctcgctgtcctccacccccatgagcacgccgtgcagctcggtgcccccttcccccagcttctcggcgcccagcccgggctcgggcagcgagcagaaggcgcacctggaagactactactggatgaccggctacccgcagcagctgaaccccgaggcgctgggcttcagccccgaggacgcggtcgaggcgctcatcagcaacagccaccagctccagggcggcttcgatggctacgcgcgcggggcgcagcagctggccgcggcggccggggccggtgccggcgcctccttgggcggcagcggcgaggagatgggccccgccgccgccgtggtgtccgccgtgatcgccgcggccgccgcgcagagcggcgcgggcccgcactaccaccaccaccaccaccacgccgccggccaccaccaccacccgacggccggcgcgcccggcgccgcgggcagcgcggccgcctcggccggtggcgctgggggcgcgggcggcggtggcccggccagcgctgggggcggcggcggcggcggcggcggcggaggcggcgggggcgcggcgggggcggggggcgccctgcacccgcaccacgccgccggcggcctgcacttcgacgaccgcttctccgacgagcagctggtgaccatgtctgtgcgcgagctgaaccggcagctgcgcggggtcagcaaggaggaggtgatccggctgaagcagaagaggcggaccctgaaaaaccgcggctatgcccagtcctgccgcttcaagagggtgcagcagagacacgtcctggagtcggagaagaaccagctgctgcagcaagtcgaccacctcaagcaggagatctccaggctggtgcgcgagagggacgcgtacaaggagaaatacgagaagttggtgagcagcggcttccgagaaaacggctcgagcagcgacaacccgtcctctcccgagtttttcatgtgagtctgacacgcgattccagctagccaccctgataagtgctccgcgggggtccggctcgggtgtgggcttgctagttctagagccatgctcgccaccacctcaccacccccacccccaccgagtttggcccccttggccccctacacacacacaaacccgcacgcacacaccacacacacacacacacacacacacacaccccacaccctgctcgagtttgtggtggtggtggctgttttaaactggggagggaatgggtgtctggctcatggattgccaatctgaaattctccataacttgctagcttgttttttttttttttttacacccccccgccccacccccggacttgcacaatgttcaatgatctcagcagagttcttcatgtgaaacgttgatcacctttgaagcctgcatcattcacatattttttcttcttcttccccttcagttcatgaactggtgttcattttctgtgtgtgtgtgtgttttattttgtttggatttttttttttaattttacttttagagcttgctgtgttgcccaccttttttccaacctccaccctcactccttctcaacccatctcttccgagatgaaagaaaaaaaaaagcaaagtttttttttcttctcctgagttcttcatgtgagattgagcttgcaaaggaaaaaaaaatgtgaaatgttatagacttgcagcgtgccgagttccatcgggttttttttttagcattgttatgctaaaatagagaaaaaaatcctcatgaaccttccacaatcaagcctgcatcaaccttctgggtgtgacttgtgagttttggccttgtgatgccaaatctgagagtttagtctgccattaaaaaaactcattctcatctcatgcattattatgcttgctactttgtcttagcaacaatgaactataactgtttcaaagactttatggaaaagagacattatattaataaaaaaaaaaagcctgcatgctggacatgtatggtataattattttttcctttttttttccttttggcttggaaatggacgttcgaagacttatagcatggcattcatacttttgttttattgcctcatgacttttttgagtttagaacaaaacagtgcaaccgtagagccttcttcccatgaaattttgcatctgctccaaaactgctttgagttactcagaacttcaacctcccaatgcactgaaggcattccttgtcaaagataccagaatgggttacacatttaacctggcaaacattgaagaactcttaatgttttctttttaataagaatgacgccccactttggggactaaaattgtgctattgccgagaagcagtctaaaatttattttttaaaaagagaaactgccccattatttttggtttgttttatttttattttatattttttggcttttggtcattgtcaaatgtggaatgctctgggtttctagtatataatttaattctagtttttataatctgttagcccagttaaaatgtatgctacagataaaggaatgttatagataaatttgaaagagttaggtctgtttagctgtagattttttaaacgattgatgcactaaattgtttactattgtgatgttaaggggggtagagtttgcaaggggactgtttaaaaaaagtagcttatacagcatgtgcttgcaacttaaatataagttgggtatgtgtagtctttgctataccactgactgtattgaaaaccaaagtattaagaggggaaacgcccctgtttatatctgtaggggtattttacattcaaaaatgtatgtttttttttcttttcaaaattaaagtatttgggactgaattgcactaagatataacctgcaagcatataatacaaaaaaaaattgcaaaactgtttagaacgctaataaaatttatgcagttataaaaatggcattactgcacagttttaagatgatgcagatttttttacagttgtattgtggtgcagaactggattttctgtaacttaaaaaaaaatccacagttttaaaggcaataatcagtaaatgttattttcagggactgacatcctgtctttaaaaagaaatgaaaagtaaatcttaccacaataaatataaaaaaatcttgtcagttacttttcttttacatattttgctgtgcaaaattgttttatatcttgagttactaactaaccacgcgtgttgttcctatgtgcttttctttcattttcaattctggttatatcaagaaaagaataatctacaataataaacggcatttttttttgattctgtactcagtttcttagtgtacagtttaactgggcccaacaacctcgttaaaagtgtaaaatgcatccttttctccagtggaaggattcctggaggaatagggagacagtaattcagggtgaaattataggctgttttttgaagtgaggaggctggccccatatactgattagcaatatttaatatagatgtaaattatgacctcatttttttctccccaaagttttcagttttcaaatgagttgagccataattgcccttggtaggaaaaacaaaacaaaacagtggaactaggcttcctgagcatggccctacacttctgatcaggagcaaagccatccatagacagaggagccggacaaatatggcgcatcagaggtggcttgcgcacatatgcattgaacggtaaagagaaacagcgcttgccttttcactaaagttgactatttttccttcttctcttacacaccgagattttcttgttagcaaggcctgacaagatttaacataaacatgacaaatcatagttgtttgttttgttttgcttttctctttaacactgaagatcatttgtcttaaataggaaaaagaaaatccactccttacttccatatttccaagtacatatctggtttaaactatgttatcaaatcatatttcaccgtgaatattcagtggagaacttctctacctggatgagctagtaatgatttcagatcatgctatccccagaaataaaagcaaaaaataatacctgtgtggaatataggctgtgctttgatttactggtatttaccccaaaataggctgtgtatgggggctgacttaaagatcccttggaaagactcaaaactaccttcactagtaggactcctaagcgctgacctatttttaaatgacacaaattcatgaaactaatgttacaaattcatgcagtttgcactcttagtcatcttcccctagcacaccaatagaatgttagacaaagccagcactgttttgaaaatacagccaaacacgatgacttttgttttgttttctgccgttcttaaaagaaaaaaagataatattgcaactctgactgaaagacttatttttaagaaaacaggttgtgtttggtgctgctaagttctggccagtttatcatctggccttcctgcctattttttacaaaacacgaagacagtgtgtaacctcgacattttgaccttcctttatgtgctagtttagacaggctcctgaatccacacttaattttgcttaacaaaagtcttaatagtaaacctcccctcatgagcttgaagtcaagtgttcttgacttcagatatttctttcctttttttttttttttcctcatcacaactaagagatacacaaactctgaagaagcagaaatggagagaatgcttttaacaaaaaagcatctgatgaaagattttaggcaaacattctcaaaataagagtgatattctggatgtagttattgcagttatctcatgacaaatgaggcctggattggaaggaaaatatagttgtgtagaattaagcattttgataggaatctacaaggtagttgaatataataagcaggtttgggcccccaaactttagaaaatcaaatgcaaaggtgctggcaaaaatgaggtttgagtggctggctgtaagagaaggttaactcctagtaaaaggcatttttagaaataacaattactgaaaactttgaagtatagtgggagtagcaaacaaatacatgttttttttttcttacaaagaactcctaaatcctgagtaagtgccattcattacaataagtctctaaatttaaaaaaaaaaaaatcatatgaggaaatctagctttcccctttacgctgcgtttgatctttgtctaaatagtgttaaaattcctttcattccaattacagaactgagcccactcgcaagttggagccatcagtgggatacgccacattttggaagccccagcatcgtgtacttaccagtgtgttcacaaaatgaaatttgtgtgagagctgtacattaaaaaaaatcatcattattattattatttgcagtcatggagaaccacctacccctgacttctgtttagtctcctttttaaataaaaattactgtgttagagaagaaggctattaaatgtagtagttaactatgcctcttgtctgggggtttcatagagaccggtaggaaagcgcactcctgcttttcgatttatggtgtgtgcaagtaaacaggtgcattgctttcaacctgccatactagttttaaaaattcactgaaattacaaagatacatatatatgcatatatataatggaaagtttcccggaatgcaacaattagcattttaaaatcatatataggcatgcacattctaaatagtactttttcatgcttcattgtttctctggcagataattttactaagaagaaaaatagatattcgactccccttccctaaacaaatccacgggcagaggctccagcggagccgagccccctggttttctcgtaggccctagacggtgttgcatttatcagtgatgtcaaacgtgctcatttgtcagacatagctgtaaatgaaaacaatgtgtggcaaaatacaaagttaaaaaaaaaa

SEQ ID NO: 4 - protein, 400 aa, Homo sapiens
MASELAMSNSDLPTSPLAMEYVNDFDLMKFEVKKEPVETDRIISQCGRLIAGGSLSSTPMSTPCSSVPPSPSFSAPSPGSGSEQKAHLEDYYWMTGYPQQLNPEALGFSPEDAVEALISNSHQLQGGFDGYARGAQQLAAAAGAGAGASLGGSGEEMGPAAAVVSAVIAAAAAQSGAGPHYHHHHHHAAGHHHHPTAGAPGAAGSAAASAGGAGGAGGGGPASAGGGGGGGGGGGGGGAAGAGGALHPHHAAGGLHFDDRFSDEQLVTMSVRELNRQLRGVSKEEVIRLKQKRRTLKNRGYAQSCRFKRVQQRHVLESEKNQLLQQVDHLKQEISRLVRERDAYKEKYEKLVSSGFRENGSSSDNPSSPEFFITEPTRKLEPSVGYATFWKPQHRVLTSV

SEQ ID NO: 5 - protein, 373 aa, Homo sapiens
MASELAMSNSDLPTSPLAMEYVNDFDLMKFEVKKEPVETDRIISQCGRLIAGGSLSSTPMSTPCSSVPPSPSFSAPSPGSGSEQKAHLEDYYWMTGYPQQLNPEALGFSPEDAVEALISNSHQLQGGFDGYARGAQQLAAAAGAGAGASLGGSGEEMGPAAAVVSAVIAAAAAQSGAGPHYHHHHHHAAGHHHHPTAGAPGAAGSAAASAGGAGGAGGGGPASAGGGGGGGGGGGGGGAAGAGGALHPHHAAGGLHFDDRFSDEQLVTMSVRELNRQLRGVSKEEVIRLKQKRRTLKNRGYAQSCRFKRVQQRHVLESEKNQLLQQVDHLKQEISRLVRERDAYKEKYEKLVSSGFRENGSSSDNPSSPEFFM

SEQ ID NO: 6 - RNA, 19 nt, Artificial Sequence
  c-MAF specific siRNA
acggcucgagcagcgacaa

SEQ ID NO: 7 - RNA, 19 nt, Artificial Sequence
  c-MAF specific siRNA
cuuaccaguguguucacaa

SEQ ID NO: 8 - RNA, 20 nt, Artificial Sequence
  c-MAF specific siRNA
uggaagacuacuacuggaug

SEQ ID NO: 9 - RNA, 20 nt, Artificial Sequence
  c-MAF specific siRNA
auuugcagucauggagaacc

SEQ ID NO: 10 - RNA, 20 nt, Artificial Sequence
  c-MAF specific siRNA
caaggagaaauacgagaagu

SEQ ID NO: 11 - RNA, 20 nt, Artificial Sequence
  c-MAF specific siRNA
acaaggagaaauacgagaag

SEQ ID NO: 12 - RNA, 20 nt, Artificial Sequence
  c-MAF specific siRNA
accuggaagacuacuacugg

SEQ ID NO: 13 - DNA, 13878 bp, Homo sapiens
aactatatattaaacacctccggtctgagaggccgtgttgggtgtctttgtcaggtgaagaaagagaagaaggctggtacaccttcccaggaattctcactgaagaaaacatctggattttttacatctcttgtgcaaaacaaacaaagatttcattaagtgatgtatattgttttccaaggaagaaacctgcagagacaaaaacaaataagcaaataattgaaacaaaaatatgataaacccccaaattcttccagtgctaatttacttgttatcatggttctctacaaaggcagagatcactaattacaggtttttccagaattcacatttcacgtcaagatcatccaatccaaacagtgtacggaaagcctagggccttcttcactttgccccctaccccaccctacacacacgcccccatctaaatgatacccttggaaagaaacctacacatctcatttgtctatattttgcttcctccctcgcctcccggtaaccaaatgtgagttgttctctaactgcactggagaatcagaatttattgtacatatgtttgtgttccacttaataaaaaaacctatattttaagataaactttgttagtaattcatgaggtaagtgactatttatgctaatcaggcagaaatatattctcaagcataatgcattacataaatttgaatgtaaaatgttcaattatgaagtaaatacaggtaatgcaaataataaattacctctaataaaaattataaaagatgtgccttgaaagagagagcggctttaacttacaactgtgaattgcttaaagagaaaagaattaataaatgctgaattactctgatgattatttagcacataattcacctattcataacgactcctagtaatcagactgttgtttcacatcctccaacatgaggcaagactgtttcctcagcaattttgcccttatcagattatctcgtctgattctattaattttcttccatgaatctgctaacagtgatttgtgatttacttaccctgctaactgaagactgttaaaaggatttatctaacactggacctaagaacagtgtacgccttatcgttcagttactctgaagaactctttctcaaatcaatttagttggtttcatagtgaaatttagtggacactggttagttctgccccataaaatcagcccctaaacaaagagtccagacaccatacctgatgcatcccattctattcagattatggatgtctgattccaacatgatatatttgagttgctataactcacaatcggggaaaatatattcctttaagcttttaatctttgtaatttggacatgaacaggggttttgtttttcatttttgcatgaagtcattatgtatgtactgacgtgaaactataattgtgtttctgatgttactgtgtcacaatattctatgcgatgtaacccatgtcctcctccccctcacaaatctcctataaatattcattgctttcaaaaactttaatactactggtccgaattggtcaataatgacaaatgcatggtttctaaattactgtatattgttctacagagattactagagtatatatagcaaggggatgttaagcagtaagaaaacacagttcacattgtatttggattagattggcttggatagaagtgaaacaaacaatgttagcaaagaagtctaaagacatgtggcccactgtaattgtacagaatcaaaaacctgaatagtactcattaaaatgagagagctcaattgttataaaagaaatgctgctaacagagaactgtaaatgtttagacacccctgtgaatcactaaataataatgtaaaaaggataaaaatgagaattaagttataagcctgagagcattactgctacacatctaaaaaaataattctgatcctctcttttttttttccaagagaaaatgggcgactataaaagaccttgcaataagagaaataaaaataccatgtcttcacagcagtgtacataaataaaccataaaaatgtgcagataataatatatttagctgcccaaacatgggcatttaatttctagaaatgatatataacaatgtaacaattagatactcagccatgaatgtgtatggcacagtcttcatcattagcaaactttgtgtataaaatattatttattatttattataatactgctttcagaggcaatgatcataccttacagcttttaacacaaatatgatgcaaaaggattaaaagtatatcataaacaaacaataaattctttctaaatacacttaaattcatattttacatgaaaaatataaacttcctacatttgtgactactgacttttaaaaagacctagaaaactattgttacgggcaatgttaaatgacataatgcttatgtaatggaaagtgtggattttcctctaaataaactataatcccttaacttcattactagggaaaatattgttaaagagaaggaaagcaagggaattctgctaggttgcataaatattgacataatcttcactctttcttccccaaactggtaatagacatagtttattccacccaacaaaatgctcttataagaccaaaactacccttattaacaacttctctgcagtcacgatgaaaagaaacactacttgtctgaaaaataccgacagcgctgcccttttcagattagggtgtgcctacgaatcttttgggaagtcttccattaaggattcctgggtttgctgaaactgaagtctactaggatcagagaaattaacacaggtctaatatggtgcaaggaacgagtgagagacacctgaggttataaatagcaaagcatgctgcggggtggggaagaccattctgaagtgcaatgttcaagacgctggcttaatatatgactaagtgtcagaagtcaggttttctgagaattactttccagataaacaactttatagcactgcacttaatcttacttactagagacatctcatttatcactgaattacaagtaactttaatcctattgatattgccataaagcccgttgaaaatccatcctggcacttttaaagggtttggggccctgttacatggggatcctcttgcaaaggtctcagccagaaattacaccccgagggtgtctgtatcccctggcctctttgtcaacaatcaaggagaagaggaggggcaaaaatgatctctgcatctgccagcactttcttcggcccctttcctatagggtcgggttctcccacttcagtcaaactaactttgtgtgtctctttcctcctcccacactgggtaaccagctgcttttcacttcatcgacaaaactggacacggatcaatttcaactgacctttgccgaaaggtggcgctgttgaggtaaaaaccaactcgctccaacaatagtttccactcttcgatccttttgcaggcttttcagaatttttttttttttttaatgcaccctcctagcgtctcccccttctcataaagtaaaataaatacgattaaaaacaccaaatgcatttcattaattgaaggaatcaacagtcccaacttctaagcagacgggctggtcttccaaaggctgggtcggtttcaggagctttctctccaaataaatctctgcttcttcgacttgcctatcgctttaaaatcttagaaacagagttagttgttggtttccttcttttttctttttcttttttatttcttttttgcataaacttttagagaatcaatctagaaatttgaactacttattagcatttgcaactgggggtggggggagcagcctcccccaccccaccccccactctgcgtttccggactagttccagaaaccgcggtttaaaatttaacccttcgagggtagctggtgagggctggggtattgtttttcccccttgctccctgccacgatcaagtccgaaataattaaaggaaacgtaaaagtgcaaagggcgcgcctgaccctgataaacagaggtcagatttcgtaaggggacgggtgagtgtgagtgtgtgtgtgtttgtgtgtgtgtgtgtaagagagagagagagcgagcgcgcaatatgagtctcaaaggccaaactccggccagtcaggagccggaaggctgagcccggctgacctgactttgagcttccccggagttatctcgcataggcgctcgctctgtccaagggcacgcgacgccagcgggcagccggtctccgtgaagaatggcctctaaacaacttattttacctcgttgtaaagagagggataaaatgggctttccctctccacggatgcccagccttctgggcaggcgcatggccgggcggcgcccagcccgcagccccgatccggacaccccactgcatccctcccttcccggtcccttccccgcacgggcgcccgagagacggacaaagagttggggccaagtttgagcgccgggcacggccaggctcagggaaggaaggtccccggcagacacctgggtaccagagttggtgcgaggaggaaaagctgggaggcgaattcacaatcctgggggtggagggcaggcaggggaggggaatcaggccaatcccagccgagtgagcccccagcgagctggggctccggatgggaggcctgtctcgcgctccaaagaaaagcaaaccgccctcccaggtccgcccggattgccgaagcccctctggaaaaactccttcccctcttacaccaaactttgcgccgggcctcgttccctcccgggtaggcagcggcgcaggaagggttaagccagcccgtcccagctgacagtcagctgattgggccctgattgacagctccgaaaagtttccttgtttctatactattatgctaatcgcggccgctctcgccgcctcccattggcccggagtgccagtcaatttctcatttggacctgacgtcacgagtgctataaaactcagcaattgctttaaactcttcttgctggatcagaggctttaaaatcttttttcatcttctagctgtagctcgggctgcttgtcggcttggcctccccctcccccctttgctctctgcctcgtctttccccaggacttcgctattttgcttttttaaaaaaaggcaagaaagaactaaactcccccctccctctcctccagtcgggctgcacctctgccttgcactttgcacagaggtagagagcgcgcgagggagagagaggaaagaaaaaaaataataaagagagccaagcagaagaggaggcgagaagcatgaagtgttaactcccccgtgccaaggcccgcgccgcccggacagacgcccgccgcgcctccagccccgagcggacgccgcgcgcgccctgcctgcagcccgggccggcgaggcgagcccttccttatgcaaagcgcgcagcggagcggcgagcgggggacgccgcgcaccgggccgggctcctccagcttcgccgccgcagccaccaccgccgccaccgcagctcgcggaggatcttcccgagcctgaagccgccggctcggcgcgcaaggaggcgagcgagcaaggaggggccggggcgagcgagggagcacattggcgtgagcaggggggagggagggcgggcgcggggggcgcgggcagggcgggggggtgtgtgtgtgagcgcgctcggaggtttcgggccagccaccgccgcgcaagctagaagcgccccagcccggcaagctggctcacccgctggccacccagcacagcccgctggcccctctcctgcagcccatctggcggagcggcggcggcggcggcggcggcggcaggagaatggcatcagaactggcaatgagcaactccgacctgcccaccagtcccctggccatggaatatgttaatgacttcgatctgatgaagtttgaagtgaaaaaggaaccggtggagaccgaccgcatcatcagccagtgcggccgtctcatcgccgggggctcgctgtcctccacccccatgagcacgccgtgcagctcggtgcccccttcccccagcttctcggcgcccagcccgggctcgggcagcgagcagaaggcgcacctggaagactactactggatgaccggctacccgcagcagctgaaccccgaggcgctgggcttcagccccgaggacgcggtcgaggcgctcatcagcaacagccaccagctccagggcggcttcgatggctacgcgcgcggggcgcagcagctggccgcggcggccggggccggtgccggcgcctccttgggcggcagcggcgaggagatgggccccgccgccgccgtggtgtccgccgtgatcgccgcggccgccgcgcagagcggcgcgggcccgcactaccaccaccaccaccaccacgccgccggccaccaccaccacccgacggccggcgcgcccggcgccgcgggcagcgcggccgcctcggccggtggcgctgggggcgcgggcggcggtggcccggccagcgctgggggcggcggcggcggcggcggcggcggaggcggcgggggcgcggcgggggcggggggcgccctgcacccgcaccacgccgccggcggcctgcacttcgacgaccgcttctccgacgagcagctggtgaccatgtctgtgcgcgagctgaaccggcagctgcgcggggtcagcaaggaggaggtgatccggctgaagcagaagaggcggaccctgaaaaaccgcggctatgcccagtcctgccgcttcaagagggtgcagcagagacacgtcctggagtcggagaagaaccagctgctgcagcaagtcgaccacctcaagcaggagatctccaggctggtgcgcgagagggacgcgtacaaggagaaatacgagaagttggtgagcagcggcttccgagaaaacggctcgagcagcgacaacccgtcctctcccgagtttttcatgtgagtctgacacgcgattccagctagccaccctgataagtgctccgcgggggtccggctcgggtgtgggcttgctagttctagagccatgctcgccaccacctcaccacccccacccccaccgagtttggcccccttggccccctacacacacacaaacccgcacgcacacaccacacacacacacacacacacacacacaccccacaccctgctcgagtttgtggtggtggtggctgttttaaactggggagggaatgggtgtctggctcatggattgccaatctgaaattctccataacttgctagcttgttttttttttttttttacacccccccgccccacccccggacttgcacaatgttcaatgatctcagcagagttcttcatgtgaaacgttgatcacctttgaagcctgcatcattcacatattttttcttcttcttccccttcagttcatgaactggtgttcattttctgtgtgtgtgtgtgttttattttgtttggatttttttttttaattttacttttagagcttgctgtgttgcccaccttttttccaacctccaccctcactccttctcaacccatctcttccgagatgaaagaaaaaaaaaagcaaagtttttttttcttctcctgagttcttcatgtgagattgagcttgcaaaggaaaaaaaaatgtgaaatgttatagacttgcagcgtgccgagttccatcgggttttttttttagcattgttatgctaaaatagagaaaaaaatcctcatgaaccttccacaatcaagcctgcatcaaccttctgggtgtgacttgtgagttttggccttgtgatgccaaatctgagagtttagtctgccattaaaaaaactcattctcatctcatgcattattatgcttgctactttgtcttagcaacaatgaactataactgtttcaaagactttatggaaaagagacattatattaataaaaaaaaaaagcctgcatgctggacatgtatggtataattattttttcctttttttttccttttggcttggaaatggacgttcgaagacttatagcatggcattcatacttttgttttattgcctcatgacttttttgagtttagaacaaaacagtgcaaccgtagagccttcttcccatgaaattttgcatctgctccaaaactgctttgagttactcagaacttcaacctcccaatgcactgaaggcattccttgtcaaagataccagaatgggttacacatttaacctggcaaacattgaagaactcttaatgttttctttttaataagaatgacgccccactttggggactaaaattgtgctattgccgagaagcagtctaaaatttattttttaaaaagagaaactgccccattatttttggtttgttttatttttattttatattttttggcttttggtcattgtcaaatgtggaatgctctgggtttctagtatataatttaattctagtttttataatctgttagcccagttaaaatgtatgctacagataaaggaatgttatagataaatttgaaagagttaggtctgtttagctgtagattttttaaacgattgatgcactaaattgtttactattgtgatgttaaggggggtagagtttgcaaggggactgtttaaaaaaagtagcttatacagcatgtgcttgcaacttaaatataagttgggtatgtgtagtctttgctataccactgactgtattgaaaaccaaagtattaagaggggaaacgcccctgtttatatctgtaggggtattttacattcaaaaatgtatgtttttttttcttttcaaaattaaagtatttgggactgaattgcactaagatataacctgcaagcatataatacaaaaaaaaattgcaaaactgtttagaacgctaataaaatttatgcagttataaaaatggcattactgcacagttttaagatgatgcagatttttttacagttgtattgtggtgcagaactggattttctgtaacttaaaaaaaaatccacagttttaaaggcaataatcagtaaatgttattttcagggactgacatcctgtctttaaaaagaaatgaaaagtaaatcttaccacaataaatataaaaaaatcttgtcagttacttttcttttacatattttgctgtgcaaaattgttttatatcttgagttactaactaaccacgcgtgttgttcctatgtgcttttctttcattttcaattctggttatatcaagaaaagaataatctacaataataaacggcatttttttttgattctgtactcagtttcttagtgtacagtttaactgggcccaacaacctcgttaaaagtgtaaaatgcatccttttctccagtggaaggattcctggaggaatagggagacagtaattcagggtgaaattataggctgttttttgaagtgaggaggctggccccatatactgattagcaatatttaatatagatgtaaattatgacctcatttttttctccccaaagttttcagttttcaaatgagttgagccataattgcccttggtaggaaaaacaaaacaaaacagtggaactaggcttcctgagcatggccctacacttctgatcaggagcaaagccatccatagacagaggagccggacaaatatggcgcatcagaggtggcttgcgcacatatgcattgaacggtaaagagaaacagcgcttgccttttcactaaagttgactatttttccttcttctcttacacaccgagattttcttgttagcaaggcctgacaagatttaacataaacatgacaaatcatagttgtttgttttgttttgcttttctctttaacactgaagatcatttgtcttaaataggaaaaagaaaatccactccttacttccatatttccaagtacatatctggtttaaactatgttatcaaatcatatttcaccgtgaatattcagtggagaacttctctacctggatgagctagtaatgatttcagatcatgctatccccagaaataaaagcaaaaaataatacctgtgtggaatataggctgtgctttgatttactggtatttaccccaaaataggctgtgtatgggggctgacttaaagatcccttggaaagactcaaaactaccttcactagtaggactcctaagcgctgacctatttttaaatgacacaaattcatgaaactaatgttacaaattcatgcagtttgcactcttagtcatcttcccctagcacaccaatagaatgttagacaaagccagcactgttttgaaaatacagccaaacacgatgacttttgttttgttttctgccgttcttaaaagaaaaaaagataatattgcaactctgactgaaagacttatttttaagaaaacaggttgtgtttggtgctgctaagttctggccagtttatcatctggccttcctgcctattttttacaaaacacgaagacagtgtgtaacctcgacattttgaccttcctttatgtgctagtttagacaggctcctgaatccacacttaattttgcttaacaaaagtcttaatagtaaacctcccctcatgagcttgaagtcaagtgttcttgacttcagatatttctttcctttttttttttttttcctcatcacaactaagagatacacaaactctgaagaagcagaaatggagagaatgcttttaacaaaaaagcatctgatgaaagattttaggcaaacattctcaaaataagagtgatattctggatgtagttattgcagttatctcatgacaaatgaggcctggattggaaggaaaatatagttgtgtagaattaagcattttgataggaatctacaaggtagttgaatataataagcaggtttgggcccccaaactttagaaaatcaaatgcaaaggtgctggcaaaaatgaggtttgagtggctggctgtaagagaaggttaactcctagtaaaaggcatttttagaaataacaattactgaaaactttgaagtatagtgggagtagcaaacaaatacatgttttttttttcttacaaagaactcctaaatcctgagtaagtgccattcattacaataagtctctaaatttaaaaaaaaaaaaatcatatgaggaaatctagctttcccctttacgctgcgtttgatctttgtctaaatagtgttaaaattcctttcattccaattacagaactgagcccactcgcaagttggagccatcagtgggatacgccacattttggaagccccagcatcgtgtacttaccagtgtgttcacaaaatgaaatttgtgtgagagctgtacattaaaaaaaatcatcattattattattatttgcagtcatggagaaccacctacccctgacttctgtttagtctcctttttaaataaaaattactgtgttagagaagaaggctattaaatgtagtagttaactatgcctcttgtctgggggtttcatagagaccggtaggaaagcgcactcctgcttttcgatttatggtgtgtgcaagtaaacaggtgcattgctttcaacctgccatactagttttaaaaattcactgaaattacaaagatacatatatatgcatatatataatggaaagtttcccggaatgcaacaattagcattttaaaatcatatataggcatgcacattctaaatagtactttttcatgcttcattgtttctctggcagataattttactaagaagaaaaatagatattcgactccccttccctaaacaaatccacgggcagaggctccagcggagccgagccccctggttttctcgtaggccctagacggtgttgcatttatcagtgatgtcaaacgtgctcatttgtcagacatagctgtaaatgaaaacaatgtgtggcaaaatacaaagttagttaaatacacaccctctgtgtgattttttgctcccttttcttttttgctcctactcaaaaaaaaaaaaatcacctcctttacatttccctggcttcttgcatgtttcccttttcaaaaaccatgtaataattttttacaatgtatctgacacattaatatattgacatcaaataggcagacattctacttttgcctggcaaataaatctgctacggagacatcatttcctcactgtctcaaagccataactacctgggagtctttcaacacagacccctccgatgggaaatgctgtttattactgaatgcaggatgctcacgctctgatcttttctcccttgtgcctttaccccagtcatttttacttagcaacaccaattctagatacttctgttctgaagtagaaccacccccttgccacactgccagttttcctgctaaaagcagtggacagaagacagatcatggtcaccctcacaaacatggcacacagctgtctcggtagctgcattcccagcatgtcctggtctaaatatctagagttgcctatgacacgttcaaaggttcccaagcacagtacattgggaggcttttgctgctgtggccgttgttttcgtttaggccaacttacttccgtattcacatactcttggctttacgaaatacactcctccagtctactaggccaatcaatatatttaaaagtctgattgccacataagtctctctctctctctttttgttttttgtttgtttgtttttttctgttttggctgccggtagttaaagactgagataggttggaagactaaaatacaggagtacatgagtgacaaccttcagccgtctgatttccatgccggtaaaacacacaaccaagctcttcttagcgctgctaatataaacattcactaagagggaataggaagtgagatttaccagcttcactttgctgatttgcaaggttccccactacgattcactgtcatttgatttttgaaaaataattttgtccgtctctttgaagaaatgtcttagttcttttattttgtttgtttggttttttttagagaagttttatctgcagtgataggctacaatttttatctccgctgattatttgtcaggatgctgaatgaataatttggtcctgtgccttccttgttgttctgaggaaaataagagaaacttggaagtttgtttcactcttagcccatcctaaatctaaaagaagatgtcccaggtccaggcaggccatgtagtagttataaaggaggtggtccaggtccagccacctcaatcaggatttgtttgttttgaagcatttgcttaaaagcggagcaagagtcttaacccaacttgccataacactgcttttctcgcttttgatgtaaatcttcaaaattcagacatcaaacagccccagaaaaggggaattctctccaggcattgctccgccccagctcctgaacaaacccagctctgtctagcatttttttccctagcgggggtaggggacagggtgagagaatttcagtctcccaggctgtctcatgattgttagggcataaagaaacacagtcctgccacaaattgggagcatctttaccctttagagagaaacaaaacaaaactaaacaaacaaatcaaattgctttgcatgaaggcgtagcaaataaaatctcgggctccctgttccctgcaccatttgtaggaggtgagaaatgagggaaacaagagaaaggggaactttaaaagcgggaggcccagaaataatccctgttaccagtctgaatttcacttgctccgtggctaacgtcagacctagtgtgcatgtatgccagaagtaaactaggctcggctgtccatttctttaaaatatgttcacatgtttcctttttgaaaacaattttggggactaaacccaaatggagagatttgaggaaatcgttaatgtcttaacatttgagtatatttataaatgtatcagtctgtgat

SEQ ID NO: 14 - protein, 455 aa, Artificial Sequence
  INB-1-11-8 (H1) Heavy Chain
  MISC_FEATURE (1)..(132): Variable Heavy Chain
  MISC_FEATURE (133)..(138): Start of constant region
  MISC_FEATURE (317)..(416): Variant
METGLRWLLLVAVLKGVQCQSLEESGGRLVTPGTPLTLTCTASGFSLNNYPMTWVRQAPGKGLDYIGVINNSGETAYATWAKRRFTISRTSTTLYLKIASPTIEDTATYFCARGGPVSSDMWGPGTLVIVSSGQPKAPSVFPLAPCCGDTPSSTVTLGCLVKGYLPEPVTVTWNSGTLTNGVRTFPSVRQSSGLYSLSSVVSVTSSSQPVTCNVAHPATNTKVDKTVAPSTCSKPTCPPPELLGGPSVFIFPPKPKDTLMISRTPEVTCVVVDVSQDDPEVQFTWYINNEQVRTARPPLREQQFNSTIRVVSTLPIAHQDWLRGKEFKCKVHNKALPAPIEKTISKARGQPLEPKVYTMGPPREELSSRSVSLTCMINGFYPSDISVEWEKNGKAEDNYKTTPAVLDSDGSYFLYSKLSVPTSEWQRGDVFTCSVMHEALHNHYTQKSISRSPGK

SEQ ID NO: 15 - protein, 132 aa, Artificial Sequence
  INB-1-11-8 (H1) Variable Heavy Chain
METGLRWLLLVAVLKGVQCQSLEESGGRLVTPGTPLTLTCTASGFSLNNYPMTWVRQAPGKGLDYIGVINNSGETAYATWAKRRFTISRTSTTLYLKIASPTIEDTATYFCARGGPVSSDMWGPGTLVIVSS

SEQ ID NO: 16 - protein, 236 aa, Artificial Sequence
  INB-1-11-8 (L4) Light Chain
  MISC_FEATURE (1)..(133): Variable Light Chain
  MISC_FEATURE (134)..(139): Start of constant region
  MISC_FEATURE (146)..(149): Variant
MDTRAPTQLLGLLLLWLPGATFAQVLTQTASPVSAVVGGTVTINCQSSQSVYRGDWLAWYQQRPGQPPKLLIYGASTLASGVPSRFKGSGSGTHFTLTISDLDCDDAATYYCAGGFSGHIYDFGGGTEVVVKGDPVAPTVLIFPPAADQVATGTVTIVCVANKYFPDVTVTWEVDGTTQTTGIENSKTPQNSADCTYNLSSTLTLTSTQYNSHKEYTCKVTQGTTSVVQSFNRGDC

SEQ ID NO: 17 - protein, 133 aa, Artificial Sequence
  INB-1-11-8 (L4) Variable Light Chain
MDTRAPTQLLGLLLLWLPGATFAQVLTQTASPVSAVVGGTVTINCQSSQSVYRGDWLAWYQQRPGQPPKLLIYGASTLASGVPSRFKGSGSGTHFTLTISDLDCDDAATYYCAGGFSGHIYDFGGGTEVVVKG

SEQ ID NO: 18 - protein, 13 aa, Artificial Sequence
  CDR1
QSSQSVYRGDWLA

SEQ ID NO: 19 - protein, 7 aa, Artificial Sequence
  CDR2
GASTLAS

SEQ ID NO: 20 - protein, 10 aa, Artificial Sequence
  CDR3
AGGFSGHIYD

SEQ ID NO: 21 - protein, 5 aa, Artificial Sequence
  CDR1
NYPMT

SEQ ID NO: 22 - protein, 16 aa, Artificial Sequence
  CDR2
VINNSGETAYATWAKR

SEQ ID NO: 23 - protein, 8 aa, Artificial Sequence
  CDR3
GGPVSSDM

SEQ ID NO: 24 - protein, 18 aa, Homo sapiens
EQKAHLEDYYWMTGYPQQ